European Patent Application EP 4 174 167 A1, published May 3, 2023. Title: New microorganism belonging to genus Lactobacillus, and control agent and control method against plant disease caused by Ralstonia solanacearum or Ralstonia pseudosolanacearum. Applicant: SUMITOMO CHEMICAL COMPANY, LIMITED. The sequence listing filed with the application follows.

SEQUENCE LISTING (5 sequences)

SEQ ID NO: 1 - DNA, 1485 bp, Lactobacillus sp. SC-2001 (NITE BP-03197)
gacgaacgctggcggcgtgcctaatacatgcaagtcgaacgcaaaactttcaccgaatgcttgcattcaccggaagttttgagtggcgaacgggtgagtaacacgtgggtaacctgcccagaagagggggataacacttggaaacaggtgctaataccgcataacaataaaaaccgcatggtttttatttaaaagatggttttgctatcacttctggatggacccgcggcgtattagctagttggtaaggtaaaggcttaccaaggcaatgatacgtagccgaactgagaggttgatcggccacattgggactgagacacggcccaaactcctacgggaggcagcagtagggaatcttccacaatggacgaaagtctgatggagcaacgccgcgtgagtgaagaaggttttcggatcgtaaaactctgttgttagagaagaacgtgtgtgagagtaactgctcatgcagtgacggtatctaaccagaaagccacggctaactacgtgccagcagccgcggtaatacgtaggtggcaagcgttgtccggatttattgggcgtaaagggaacgcaggcggttttttaagtctgatgtgaaagccttcggcttaaccgaagtcatgcattggaaactgaaagacttgagtgcagaagaggagagtggaactccatgtgtagcggtgaaatgcgtagatatatggaagaacaccagtggcgaaagcggctctctggtctgtaactgacgctgaggttcgaaagtgtgggtagcaaacaggattagataccctggtagtccacaccgtaaacgatgaatgctaagtgttggagggtttccgcccttcggtgctgcagctaacgcattaagcattccgcctggggagtacgaccgcaaggttgaaactcaaaggaattgacgggggcccgcacaagcggtggagcatgtggtttaattcgaagcaacgcgaagaaccttaccaggtcttgacatcttctgacaacctaagagattaggtgttcccttcggggacagaatgacaggtggtgcatggttgtcgtcagctcgtgtcgtgagatgttgggttaagtcccgcaacgagcgcaacccttattattagttgccagcattaagttgggcactctagtgagactgccggtgacaaaccggaggaaggtggggatgacgtcaaatcatcatgccccttatgacctgggctacacacgtgctacaatggacggtacaacgagtcgcgaaaccgcgaggtttagctaatctcttaaagccgttctcagttcggattgtaggctgcaactcgcctacatgaagtcggaatcgctagtaatcgcggatcagcatgccgcggtgaatacgttcccgggccttgtacacaccgcccgtcacaccatgagagtttgtaacacccaaagccggtgaggtaacctttatggaaccagccgtctaaggtgggacagatgattggggtgaag

SEQ ID NO: 2 - DNA, 22 bp, Artificial Sequence
  PCR primer 759
gtcgccgtcaactcaactttcc

SEQ ID NO: 3 - DNA, 24 bp, Artificial Sequence
  PCR primer 760
gtcgccgtcagcaatgcggaatcg

SEQ ID NO: 4 - DNA, 21 bp, Artificial Sequence
  PCR primer Nmult21:1F
cgttgatgaggcgcgcaattt

SEQ ID NO: 5 - DNA, 22 bp, Artificial Sequence
  PCR primer Nmult21:RR
ttcgcttgaccctataacgagt